European Patent Specification EP 3 547 831 B1, published April 1, 2026. Title: HUMANIZED MOUSE MODEL WITH IMPROVED HUMAN INNATE IMMUNE CELL DEVELOPMENT. Applicant: The Jackson Laboratory. The sequence listing filed with the application follows.

SEQUENCE LISTING (25 sequences)

SEQ ID NO: 1 - DNA, 1662 bp, Homo sapiens
atgaccgcgccgggcgccgccgggcgctgccctcccacgacatggctgggctccctgctgttgttggtctgtctcctggcgagcaggagtatcaccgaggaggtgtcggagtactgtagccacatgattgggagtggacacctgcagtctctgcagcggctgattgacagtcagatggagacctcgtgccaaattacatttgagtttgtagaccaggaacagttgaaagatccagtgtgctaccttaagaaggcatttctcctggtacaagacataatggaggacaccatgcgcttcagagataacacccccaatgccatcgccattgtgcagctgcaggaactctctttgaggctgaagagctgcttcaccaaggattatgaagagcatgacaaggcctgcgtccgaactttctatgagacacctctccagttgctggagaaggtcaagaatgtctttaatgaaacaaagaatctccttgacaaggactggaatattttcagcaagaactgcaacaacagctttgctgaatgctccagccaagatgtggtgaccaagcctgattgcaactgcctgtaccccaaagccatccctagcagtgacccggcctctgtctcccctcatcagcccctcgccccctccatggcccctgtggctggcttgacctgggaggactctgagggaactgagggcagctccctcttgcctggtgagcagcccctgcacacagtggatccaggcagtgccaagcagcggccacccaggagcacctgccagagctttgagccgccagagaccccagttgtcaaggacagcaccatcggtggctcaccacagcctcgcccctctgtcggggccttcaaccccgggatggaggatattcttgactctgcaatgggcactaattgggtcccagaagaagcctctggagaggccagtgagattcccgtaccccaagggacagagctttccccctccaggccaggagggggcagcatgcagacagagcccgccagacccagcaacttcctctcagcatcttctccactccctgcatcagcaaagggccaacagccggcagatgtaactggtaccgccttgcccagggtgggccccgtgaggcccactggccaggactggaatcacaccccccagaagacagaccatccatctgccctgctcagagaccccccggagccaggctctcccaggatctcatcactgcgcccccagggcctcagcaacccctccaccctctctgctcagccacagctttccagaagccactcctcgggcagcgtgctgccccttggggagctggagggcaggaggagcaccagggatcggaggagccccgcagagccagaaggaggaccagcaagtgaaggggcagccaggcccctgccccgttttaactccgttcctttgactgacacaggccatgagaggcagtccgagggatcctccagcccgcagctccaggagtctgtcttccacctgctggtgcccagtgtcatcctggtcttgctggccgtcggaggcctcttgttctacaggtggaggcggcggagccatcaagagcctcagagagcggattctcccttggagcaaccagagggcagccccctgactcaggatgacagacaggtggaactgccagtg

SEQ ID NO: 2 - DNA, 1314 bp, Homo sapiens
atgaccgcgccgggcgccgccgggcgctgccctcccacgacatggctgggctccctgctgttgttggtctgtctcctggcgagcaggagtatcaccgaggaggtgtcggagtactgtagccacatgattgggagtggacacctgcagtctctgcagcggctgattgacagtcagatggagacctcgtgccaaattacatttgagtttgtagaccaggaacagttgaaagatccagtgtgctaccttaagaaggcatttctcctggtacaagacataatggaggacaccatgcgcttcagagataacacccccaatgccatcgccattgtgcagctgcaggaactctctttgaggctgaagagctgcttcaccaaggattatgaagagcatgacaaggcctgcgtccgaactttctatgagacacctctccagttgctggagaaggtcaagaatgtctttaatgaaacaaagaatctccttgacaaggactggaatattttcagcaagaactgcaacaacagctttgctgaatgctccagccaagatgtggtgaccaagcctgattgcaactgcctgtaccccaaagccatccctagcagtgacccggcctctgtctcccctcatcagcccctcgccccctccatggcccctgtggctggcttgacctgggaggactctgagggaactgagggcagctccctcttgcctggtgagcagcccctgcacacagtggatccaggcagtgccaagcagcggccacccaggagcacctgccagagctttgagccgccagagaccccagttgtcaaggacagcaccatcggtggctcaccacagcctcgcccctctgtcggggccttcaaccccgggatggaggatattcttgactctgcaatgggcactaattgggtcccagaagaagcctctggagaggccagtgagattcccgtaccccaagggacagagctttccccctccaggccaggagggggcagcatgcagacagagcccgccagacccagcaacttcctctcagcatcttctccactccctgcatcagcaaagggccaacagccggcagatgtaactggccatgagaggcagtccgagggatcctccagcccgcagctccaggagtctgtcttccacctgctggtgcccagtgtcatcctggtcttgctggccgtcggaggcctcttgttctacaggtggaggcggcggagccatcaagagcctcagagagcggattctcccttggagcaaccagagggcagccccctgactcaggatgacagacaggtggaactgccagtg

SEQ ID NO: 3 - DNA, 619 bp, Homo sapiens
atgaccgcgccgggcgccgccgggcgctgccctcccacgacatggctgggctccctgctgttgttggtctgtctcctggcgagcaggagtatcaccgaggaggtgtcggagtactgtagccacatgattgggagtggacacctgcagtctctgcagcggctgattgacagtcagatggagacctcgtgccaaattacatttgagtttgtagaccaggaacagttgaaagatccagtgtgctaccttaagaaggcatttctcctggtacaagacataatggaggacaccatgcgcttcagagataacacccccaatgccatcgccattgtgcagctgcaggaactctctttgaggctgaagagctgcttcaccaaggattatgaagagcatgacaaggcctgcgtccgaactttctatgagacacctctccagttgctggagaaggtcaagaatgtctttaatgaaacaaagaatctccttgacaaggactggaatattttcagcaagaactgcaacaacagctttgctgaatgctccagccaaggccatgagaggcagtccgagggatcctccagcccgcagctccaggagtctgtcttccacctgctggtgcccagtg

SEQ ID NO: 4 - DNA, 1662 bp, Homo sapiens; identical to SEQ ID NO: 1

SEQ ID NO: 5 - protein, 554 aa, Homo sapiens
MTAPGAAGRCPPTTWLGSLLLLVCLLASRSITEEVSEYCSHMIGSGHLQSLQRLIDSQMETSCQITFEFVDQEQLKDPVCYLKKAFLLVQDIMEDTMRFRDNTPNAIAIVQLQELSLRLKSCFTKDYEEHDKACVRTFYETPLQLLEKVKNVFNETKNLLDKDWNIFSKNCNNSFAECSSQDVVTKPDCNCLYPKAIPSSDPASVSPHQPLAPSMAPVAGLTWEDSEGTEGSSLLPGEQPLHTVDPGSAKQRPPRSTCQSFEPPETPVVKDSTIGGSPQPRPSVGAFNPGMEDILDSAMGTNWVPEEASGEASEIPVPQGTELSPSRPGGGSMQTEPARPSNFLSASSPLPASAKGQQPADVTGTALPRVGPVRPTGQDWNHTPQKTDHPSALLRDPPEPGSPRISSLRPQGLSNPSTLSAQPQLSRSHSSGSVLPLGELEGRRSTRDRRSPAEPEGGPASEGAARPLPRFNSVPLTDTGHERQSEGSSSPQLQESVFHLLVPSVILVLLAVGGLLFYRWRRRSHQEPQRADSPLEQPEGSPLTQDDRQVELPV

SEQ ID NO: 6 - protein, 522 aa, Homo sapiens
EEVSEYCSHMIGSGHLQSLQRLIDSQMETSCQITFEFVDQEQLKDPVCYLKKAFLLVQDIMEDTMRFRDNTPNAIAIVQLQELSLRLKSCFTKDYEEHDKACVRTFYETPLQLLEKVKNVFNETKNLLDKDWNIFSKNCNNSFAECSSQDVVTKPDCNCLYPKAIPSSDPASVSPHQPLAPSMAPVAGLTWEDSEGTEGSSLLPGEQPLHTVDPGSAKQRPPRSTCQSFEPPETPVVKDSTIGGSPQPRPSVGAFNPGMEDILDSAMGTNWVPEEASGEASEIPVPQGTELSPSRPGGGSMQTEPARPSNFLSASSPLPASAKGQQPADVTGTALPRVGPVRPTGQDWNHTPQKTDHPSALLRDPPEPGSPRISSLRPQGLSNPSTLSAQPQLSRSHSSGSVLPLGELEGRRSTRDRRSPAEPEGGPASEGAARPLPRFNSVPLTDTGHERQSEGSSSPQLQESVFHLLVPSVILVLLAVGGLLFYRWRRRSHQEPQRADSPLEQPEGSPLTQDDRQVELPV

SEQ ID NO: 7 - protein, 438 aa, Homo sapiens
MTAPGAAGRCPPTTWLGSLLLLVCLLASRSITEEVSEYCSHMIGSGHLQSLQRLIDSQMETSCQITFEFVDQEQLKDPVCYLKKAFLLVQDIMEDTMRFRDNTPNAIAIVQLQELSLRLKSCFTKDYEEHDKACVRTFYETPLQLLEKVKNVFNETKNLLDKDWNIFSKNCNNSFAECSSQDVVTKPDCNCLYPKAIPSSDPASVSPHQPLAPSMAPVAGLTWEDSEGTEGSSLLPGEQPLHTVDPGSAKQRPPRSTCQSFEPPETPVVKDSTIGGSPQPRPSVGAFNPGMEDILDSAMGTNWVPEEASGEASEIPVPQGTELSPSRPGGGSMQTEPARPSNFLSASSPLPASAKGQQPADVTGHERQSEGSSSPQLQESVFHLLVPSVILVLLAVGGLLFYRWRRRSHQEPQRADSPLEQPEGSPLTQDDRQVELPV

SEQ ID NO: 8 - protein, 406 aa, Homo sapiens
EEVSEYCSHMIGSGHLQSLQRLIDSQMETSCQITFEFVDQEQLKDPVCYLKKAFLLVQDIMEDTMRFRDNTPNAIAIVQLQELSLRLKSCFTKDYEEHDKACVRTFYETPLQLLEKVKNVFNETKNLLDKDWNIFSKNCNNSFAECSSQDVVTKPDCNCLYPKAIPSSDPASVSPHQPLAPSMAPVAGLTWEDSEGTEGSSLLPGEQPLHTVDPGSAKQRPPRSTCQSFEPPETPVVKDSTIGGSPQPRPSVGAFNPGMEDILDSAMGTNWVPEEASGEASEIPVPQGTELSPSRPGGGSMQTEPARPSNFLSASSPLPASAKGQQPADVTGHERQSEGSSSPQLQESVFHLLVPSVILVLLAVGGLLFYRWRRRSHQEPQRADSPLEQPEGSPLTQDDRQVELPV

SEQ ID NO: 9 - protein, 256 aa, Homo sapiens
MTAPGAAGRCPPTTWLGSLLLLVCLLASRSITEEVSEYCSHMIGSGHLQSLQRLIDSQMETSCQITFEFVDQEQLKDPVCYLKKAFLLVQDIMEDTMRFRDNTPNAIAIVQLQELSLRLKSCFTKDYEEHDKACVRTFYETPLQLLEKVKNVFNETKNLLDKDWNIFSKNCNNSFAECSSQGHERQSEGSSSPQLQESVFHLLVPSVILVLLAVGGLLFYRWRRRSHQEPQRADSPLEQPEGSPLTQDDRQVELPV

SEQ ID NO: 10 - protein, 224 aa, Homo sapiens
EEVSEYCSHMIGSGHLQSLQRLIDSQMETSCQITFEFVDQEQLKDPVCYLKKAFLLVQDIMEDTMRFRDNTPNAIAIVQLQELSLRLKSCFTKDYEEHDKACVRTFYETPLQLLEKVKNVFNETKNLLDKDWNIFSKNCNNSFAECSSQGHERQSEGSSSPQLQESVFHLLVPSVILVLLAVGGLLFYRWRRRSHQEPQRADSPLEQPEGSPLTQDDRQVELPV

SEQ ID NO: 11 - protein, 245 aa, Homo sapiens
MKKTQTWILTCIYLQLLLFNPLVKTEGICRNRVTNNVKDVTKLVANLPKDYMITLKYVPGMDVLPSHCWISEMVVQLSDSLTDLLDKFSNISEGLSNYSIIDKLVNIVDDLVECVKENSSKDLKKSFKSPEPRLFTPEEFFRIFNRSIDAFKDFVVASETSDCVVSSTLSPEKGKAKNPPGDSSLHWAAMALPALFSLIIGFAFGALYWKKRQPSLTRAVENIQINEEDNEISMLQEKEREFQEV

SEQ ID NO: 12 - DNA, 738 bp, Homo sapiens
atgaagaagacacaaacttggattctcacttgcatttatcttcagctgctcctatttaatcctctcgtcaaaactgaagggatctgcaggaatcgtgtgactaataatgtaaaagacgtcactaaattggtggcaaatcttccaaaagactacatgataaccctcaaatatgtccccgggatggatgttttgccaagtcattgttggataagcgagatggtagtacaattgtcagacagcttgactgatcttctggacaagttttcaaatatttctgaaggcttgagtaattattccatcatagacaaacttgtgaatatagtggatgaccttgtggagtgcgtgaaagaaaactcatctaaggatctaaaaaaatcattcaagagcccagaacccaggctctttactcctgaagaattctttagaatttttaatagatccattgatgccttcaaggactttgtagtggcatctgaaactagtgattgtgtggtttcttcaacattaagtcctgagaaagggaaggccaaaaatccccctggagactccagcctacactgggcagccatggcattgccagcattgttttctcttataattggctttgcttttggagccttatactggaagaagagacagccaagtcttacaagggcagttgaaaatatacaaattaatgaagaggataatgagataagtatgttgcaagagaaagagagagagtttcaagaagtgtaa

SEQ ID NO: 13 - protein, 273 aa, Homo sapiens
MKKTQTWILTCIYLQLLLFNPLVKTEGICRNRVTNNVKDVTKLVANLPKDYMITLKYVPGMDVLPSHCWISEMVVQLSDSLTDLLDKFSNISEGLSNYSIIDKLVNIVDDLVECVKENSSKDLKKSFKSPEPRLFTPEEFFRIFNRSIDAFKDFVVASETSDCVVSSTLSPEKDSRVSVTKPFMLPPVAASSLRNDSSSSNRKAKNPPGDSSLHWAAMALPALFSLIIGFAFGALYWKKRQPSLTRAVENIQINEEDNEISMLQEKEREFQEV

SEQ ID NO: 14 - DNA, 822 bp, Homo sapiens
atgaagaagacacaaacttggattctcacttgcatttatcttcagctgctcctatttaatcctctcgtcaaaactgaagggatctgcaggaatcgtgtgactaataatgtaaaagacgtcactaaattggtggcaaatcttccaaaagactacatgataaccctcaaatatgtccccgggatggatgttttgccaagtcattgttggataagcgagatggtagtacaattgtcagacagcttgactgatcttctggacaagttttcaaatatttctgaaggcttgagtaattattccatcatagacaaacttgtgaatatagtggatgaccttgtggagtgcgtgaaagaaaactcatctaaggatctaaaaaaatcattcaagagcccagaacccaggctctttactcctgaagaattctttagaatttttaatagatccattgatgccttcaaggactttgtagtggcatctgaaactagtgattgtgtggtttcttcaacattaagtcctgagaaagattccagagtcagtgtcacaaaaccatttatgttaccccctgttgcagccagctcccttaggaatgacagcagtagcagtaataggaaggccaaaaatccccctggagactccagcctacactgggcagccatggcattgccagcattgttttctcttataattggctttgcttttggagccttatactggaagaagagacagccaagtcttacaagggcagttgaaaatatacaaattaatgaagaggataatgagataagtatgttgcaagagaaagagagagagtttcaagaagtgtaa

SEQ ID NO: 15 - DNA, 1405 bp, Homo sapiens
ccgcctcgcgccgagactagaagcgctgcgggaagcagggacagtggagagggcgctgcgctcgggctacccaatgcgtggactatctgccgccgctgttcgtgcaatatgctggagctccagaacagctaaacggagtcgccacaccactgtttgtgctggatcgcagcgctgcctttccttatgaagaagacacaaacttggattctcacttgcatttatcttcagctgctcctatttaatcctctcgtcaaaactgaagggatctgcaggaatcgtgtgactaataatgtaaaagacgtcactaaattggtggcaaatcttccaaaagactacatgataaccctcaaatatgtccccgggatggatgttttgccaagtcattgttggataagcgagatggtagtacaattgtcagacagcttgactgatcttctggacaagttttcaaatatttctgaaggcttgagtaattattccatcatagacaaacttgtgaatatagtggatgaccttgtggagtgcgtgaaagaaaactcatctaaggatctaaaaaaatcattcaagagcccagaacccaggctctttactcctgaagaattctttagaatttttaatagatccattgatgccttcaaggactttgtagtggcatctgaaactagtgattgtgtggtttcttcaacattaagtcctgagaaagattccagagtcagtgtcacaaaaccatttatgttaccccctgttgcagccagctcccttaggaatgacagcagtagcagtaataggaaggccaaaaatccccctggagactccagcctacactgggcagccatggcattgccagcattgttttctcttataattggctttgcttttggagccttatactggaagaagagacagccaagtcttacaagggcagttgaaaatatacaaattaatgaagaggataatgagataagtatgttgcaagagaaagagagagagtttcaagaagtgtaaattgtggcttgtatcaacactgttactttcgtacattggctggtaacagttcatgtttgcttcataaatgaagcagctttaaacaaattcatattctgtctggagtgacagaccacatctttatctgttcttgctacccatgactttatatggatgattcagaaattggaacagaatgttttactgtgaaactggcactgaattaatcatctataaagaagaacttgcatggagcaggactctattttaaggactgcgggacttgggtctcatttagaacttgcagctgatgttggaagagaaagcacgtgtctcagactgcatgtaccatttgcatggctccagaaatgtctaaatgctgaaaaaacacctagctttattcttcagatacaaactgcag

SEQ ID NO: 16 - protein, 189 aa, Homo sapiens
MKKTQTWILTCIYLQLLLFNPLVKTEGICRNRVTNNVKDVTKLVANLPKDYMITLKYVPGMDVLPSHCWISEMVVQLSDSLTDLLDKFSNISEGLSNYSIIDKLVNIVDDLVECVKENSSKDLKKSFKSPEPRLFTPEEFFRIFNRSIDAFKDFVVASETSDCVVSSTLSPEKDSRVSVTKPFMLPPVA

SEQ ID NO: 17 - DNA, 567 bp, Homo sapiens
atgaagaagacacaaacttggattctcacttgcatttatcttcagctgctcctatttaatcctctcgtcaaaactgaagggatctgcaggaatcgtgtgactaataatgtaaaagacgtcactaaattggtggcaaatcttccaaaagactacatgataaccctcaaatatgtccccgggatggatgttttgccaagtcattgttggataagcgagatggtagtacaattgtcagacagcttgactgatcttctggacaagttttcaaatatttctgaaggcttgagtaattattccatcatagacaaacttgtgaatatagtggatgaccttgtggagtgcgtgaaagaaaactcatctaaggatctaaaaaaatcattcaagagcccagaacccaggctctttactcctgaagaattctttagaatttttaatagatccattgatgccttcaaggactttgtagtggcatctgaaactagtgattgtgtggtttcttcaacattaagtcctgagaaagattccagagtcagtgtcacaaaaccatttatgttaccccctgttgca

SEQ ID NO: 18 - protein, 144 aa, Homo sapiens
MWLQSLLLLGTVACSISAPARSPSPSTQPWEHVNAIQEARRLLNLSRDTAAEMNETVEVISEMFDLQEPTCLQTRLELYKQGLRGSLTKLKGPLTMMASHYKQHCPPTPETSCATQIITFESFKENLKDFLLVIPFDCWEPVQE

SEQ ID NO: 19 - DNA, 435 bp, Homo sapiens
atgtggctgcagagcctgctgctcttgggcactgtggcctgcagcatctctgcacccgcccgctcgcccagccccagcacgcagccctgggagcatgtgaatgccatccaggaggcccggcgtctcctgaacctgagtagagacactgctgctgagatgaatgaaacagtagaagtcatctcagaaatgtttgacctccaggagccgacctgcctacagacccgcctggagctgtacaagcagggcctgcggggcagcctcaccaagctcaagggccccttgaccatgatggccagccactacaagcagcactgccctccaaccccggaaacttcctgtgcaacccagattatcacctttgaaagtttcaaagagaacctgaaggactttctgcttgtcatcccctttgactgctgggagccagtccaggagtga

SEQ ID NO: 20 - protein, 127 aa, Homo sapiens [sequence omitted]

SEQ ID NO: 21 - DNA, 352 bp, Homo sapiens
gccctgggagcatgtgaatgccatccaggaggcccggcgtctcctgaacctgagtagagacactgctgctgagatgaatgaaacagtagaagtcatctcagaaatgtttgacctccaggagccgacctgcctacagacccgcctggagctgtacaagcagggcctgcggggcagcctcaccaagctcaagggccccttgaccatgatggccagccactacaagcagcactgccctccaaccccggaaacttcctgtgcaacccagattatcacctttgaaagtttcaaagagaacctgaaggactttctgcttgtcatcccctttgactgctgggagccagtccaggagtga

SEQ ID NO: 22 - protein, 152 aa, Homo sapiens
MSRLPVLLLLQLLVRPGLQAPMTQTTPLKTSWVNCSNMIDEIITHLKQPPLPLLDFNNLNGEDQDILMENNLRRPNLEAFNRAVKSLQNASAIESILKNLLPCLPLATAAPTRHPIHIKDGDWNEFRRKLTFYLKTLENAQAQQTTLSLAIF

SEQ ID NO: 23 - DNA, 459 bp, Homo sapiens
atgagccgcctgcccgtcctgctcctgctccaactcctggtccgccccggactccaagctcccatgacccagacaacgcccttgaagacaagctgggttaactgctctaacatgatcgatgaaattataacacacttaaagcagccacctttgcctttgctggacttcaacaacctcaatggggaagaccaagacattctgatggaaaataaccttcgaaggccaaacctggaggcattcaacagggctgtcaagagtttacagaacgcatcagcaattgagagcattcttaaaaatctcctgccatgtctgcccctggccacggccgcacccacgcgacatccaatccatatcaaggacggtgactggaatgaattccggaggaaactgacgttctatctgaaaacccttgagaatgcgcaggctcaacagacgactttgagcctcgcgatcttttga

SEQ ID NO: 24 - protein, 133 aa, Homo sapiens
APMTQTTPLKTSWVNCSNMIDEIITHLKQPPLPLLDFNNLNGEDQDILMENNLRRPNLEAFNRAVKSLQNASAIESILKNLLPCLPLATAAPTRHPIHIKDGDWNEFRRKLTFYLKTLENAQAQQTTLSLAIF

SEQ ID NO: 25 - DNA, 402 bp, Homo sapiens
gctcccatgacccagacaacgcccttgaagacaagctgggttaactgctctaacatgatcgatgaaattataacacacttaaagcagccacctttgcctttgctggacttcaacaacctcaatggggaagaccaagacattctgatggaaaataaccttcgaaggccaaacctggaggcattcaacagggctgtcaagagtttacagaacgcatcagcaattgagagcattcttaaaaatctcctgccatgtctgcccctggccacggccgcacccacgcgacatccaatccatatcaaggacggtgactggaatgaattccggaggaaactgacgttctatctgaaaacccttgagaatgcgcaggctcaacagacgactttgagcctcgcgatcttttga